European Patent Application EP 4 253 420 A1, published October 4, 2023. Title: HER2-targeting drug. Applicant: ONO PHARMACEUTICAL CO., LTD. TOHOKU UNIVERSITY. The sequence listing filed with the application follows.

SEQUENCE LISTING (206 sequences)

SEQ ID NO: 1 - DNA, 4473 bp, Homo sapiens
aaggggaggtaaccctggcccctttggtcggggccccgggcagccgcgcgccccttcccacggggccctttactgcgccgcgcgcccggcccccacccctcgcagcaccccgcgccccgcgccctcccagccgggtccagccggagccatggggccggagccgcagtgagcaccatggagctggcggccttgtgccgctgggggctcctcctcgccctcttgccccccggagccgcgagcacccaagtgtgcaccggcacagacatgaagctgcggctccctgccagtcccgagacccacctggacatgctccgccacctctaccagggctgccaggtggtgcagggaaacctggaactcacctacctgcccaccaatgccagcctgtccttcctgcaggatatccaggaggtgcagggctacgtgctcatcgctcacaaccaagtgaggcaggtcccactgcagaggctgcggattgtgcgaggcacccagctctttgaggacaactatgccctggccgtgctagacaatggagacccgctgaacaataccacccctgtcacaggggcctccccaggaggcctgcgggagctgcagcttcgaagcctcacagagatcttgaaaggaggggtcttgatccagcggaacccccagctctgctaccaggacacgattttgtggaaggacatcttccacaagaacaaccagctggctctcacactgatagacaccaaccgctctcgggcctgccacccctgttctccgatgtgtaagggctcccgctgctggggagagagttctgaggattgtcagagcctgacgcgcactgtctgtgccggtggctgtgcccgctgcaaggggccactgcccactgactgctgccatgagcagtgtgctgccggctgcacgggccccaagcactctgactgcctggcctgcctccacttcaaccacagtggcatctgtgagctgcactgcccagccctggtcacctacaacacagacacgtttgagtccatgcccaatcccgagggccggtatacattcggcgccagctgtgtgactgcctgtccctacaactacctttctacggacgtgggatcctgcaccctcgtctgccccctgcacaaccaagaggtgacagcagaggatggaacacagcggtgtgagaagtgcagcaagccctgtgcccgagtgtgctatggtctgggcatggagcacttgcgagaggtgagggcagttaccagtgccaatatccaggagtttgctggctgcaagaagatctttgggagcctggcatttctgccggagagctttgatggggacccagcctccaacactgccccgctccagccagagcagctccaagtgtttgagactctggaagagatcacaggttacctatacatctcagcatggccggacagcctgcctgacctcagcgtcttccagaacctgcaagtaatccggggacgaattctgcacaatggcgcctactcgctgaccctgcaagggctgggcatcagctggctggggctgcgctcactgagggaactgggcagtggactggccctcatccaccataacacccacctctgcttcgtgcacacggtgccctgggaccagctctttcggaacccgcaccaagctctgctccacactgccaaccggccagaggacgagtgtgtgggcgagggcctggcctgccaccagctgtgcgcccgagggcactgctggggtccagggcccacccagtgtgtcaactgcagccagttccttcggggccaggagtgcgtggaggaatgccgagtactgcaggggctccccagggagtatgtgaatgccaggcactgtttgccgtgccaccctgagtgtcagccccagaatggctcagtgacctgttttggaccggaggctgaccagtgtgtggcctgtgcccactataaggaccctcccttctgcgtggcccgctgccccagcggtgtgaaacctgacctctcctacatgcccatctggaagtttccagatgaggagggcgcatgccagccttgccccatcaactgcacccactcctgtgtggacctggatgacaagggctgccccgccgagcagagagccagccctctgacgtccatcatctctgcggtggttggcattctgctggtcgtggtcttgggggtggtctttgggatcctcatcaagcgacggcagcagaagatccggaagtacacgatgcggagactgctgcaggaaacggagctggtggagccgctgacacctagcggagcgatgcccaaccaggcgcagatgcggatcctgaaagagacggagctgaggaaggtgaaggtgcttggatctggcgcttttggcacagtctacaagggcatctggatccctgatggggagaatgtgaaaattccagtggccatcaaagtgttgagggaaaacacatcccccaaagccaacaaagaaatcttagacgaagcatacgtgatggctggtgtgggctccccatatgtctcccgccttctgggcatctgcctgacatccacggtgcagctggtgacacagcttatgccctatggctgcctcttagaccatgtccgggaaaaccgcggacgcctgggctcccaggacctgctgaactggtgtatgcagattgccaaggggatgagctacctggaggatgtgcggctcgtacacagggacttggccgctcggaacgtgctggtcaagagtcccaaccatgtcaaaattacagacttcgggctggctcggctgctggacattgacgagacagagtaccatgcagatgggggcaaggtgcccatcaagtggatggcgctggagtccattctccgccggcggttcacccaccagagtgatgtgtggagttatggtgtgactgtgtgggagctgatgacttttggggccaaaccttacgatgggatcccagcccgggagatccctgacctgctggaaaagggggagcggctgccccagccccccatctgcaccattgatgtctacatgatcatggtcaaatgttggatgattgactctgaatgtcggccaagattccgggagttggtgtctgaattctcccgcatggccagggacccccagcgctttgtggtcatccagaatgaggacttgggcccagccagtcccttggacagcaccttctaccgctcactgctggaggacgatgacatgggggacctggtggatgctgaggagtatctggtaccccagcagggcttcttctgtccagaccctgccccgggcgctgggggcatggtccaccacaggcaccgcagctcatctaccaggagtggcggtggggacctgacactagggctggagccctctgaagaggaggcccccaggtctccactggcaccctccgaaggggctggctccgatgtatttgatggtgacctgggaatgggggcagccaaggggctgcaaagcctccccacacatgaccccagccctctacagcggtacagtgaggaccccacagtacccctgccctctgagactgatggctacgttgcccccctgacctgcagcccccagcctgaatatgtgaaccagccagatgttcggccccagcccccttcgccccgagagggccctctgcctgctgcccgacctgctggtgccactctggaaaggcccaagactctctccccagggaagaatggggtcgtcaaagacgtttttgcctttgggggtgccgtggagaaccccgagtacttgacaccccagggaggagctgcccctcagccccaccctcctcctgccttcagcccagccttcgacaacctctattactgggaccaggacccaccagagcggggggctccacccagcaccttcaaagggacacctacggcagagaacccagagtacctgggtctggacgtgccagtgtgaaccagaaggccaagtccgcagaagccctgatgtgtcctcagggagcagggaaggcctgacttctgctggcatcaagaggtgggagggccctccgaccacttccaggggaacctgccatgccaggaacctgtcctaaggaaccttccttcctgcttgagttcccagatggctggaaggggtccagcctcgttggaagaggaacagcactggggagtctttgtggattctgaggccctgcccaatgagactctagggtccagtggatgccacagcccagcttggccctttccttccagatcctgggtactgaaagccttagggaagctggcctgagaggggaagcggccctaagggagtgtctaagaacaaaagcgacccattcagagactgtccctgaaacctagtactgccccccatgaggaaggaacagcaatggtgtcagtatccaggctttgtacagagtgcttttctgtttagtttttactttttttgttttgtttttttaaagatgaaataaagacccagggggag

SEQ ID NO: 2 - protein, 1255 aa, Homo sapiens [sequence omitted]

SEQ ID NO: 3 - protein, 630 aa, Artificial Sequence
  HER2ec
TQVCTGTDMKLRLPASPETHLDMLRHLYQGCQVVQGNLELTYLPTNASLSFLQDIQEVQGYVLIAHNQVRQVPLQRLRIVRGTQLFEDNYALAVLDNGDPLNNTTPVTGASPGGLRELQLRSLTEILKGGVLIQRNPQLCYQDTILWKDIFHKNNQLALTLIDTNRSRACHPCSPMCKGSRCWGESSEDCQSLTRTVCAGGCARCKGPLPTDCCHEQCAAGCTGPKHSDCLACLHFNHSGICELHCPALVTYNTDTFESMPNPEGRYTFGASCVTACPYNYLSTDVGSCTLVCPLHNQEVTAEDGTQRCEKCSKPCARVCYGLGMEHLREVRAVTSANIQEFAGCKKIFGSLAFLPESFDGDPASNTAPLQPEQLQVFETLEEITGYLYISAWPDSLPDLSVFQNLQVIRGRILHNGAYSLTLQGLGISWLGLRSLRELGSGLALIHHNTHLCFVHTVPWDQLFRNPHQALLHTANRPEDECVGEGLACHQLCARGHCWGPGPTQCVNCSQFLRGQECVEECRVLQGLPREYVNARHCLPCHPECQPQNGSVTCFGPEADQCVACAHYKDPPFCVARCPSGVKPDLSYMPIWKFPDEEGACQPCPINCTHSCVDLDDKGCPAEQRASPLT

SEQ ID NO: 4 - DNA, 35 bp, Artificial Sequence
  InF.HindIII-H2-214H
cggtatcgataagcttgatatggacaggcttactt

SEQ ID NO: 5 - DNA, 35 bp, Artificial Sequence
  InF.HindIII-H2-250H
cggtatcgataagcttaacatgaacttagggctca

SEQ ID NO: 6 - DNA, 34 bp, Artificial Sequence
  InFr.IgG1terNotI
tctagagtcgcggccgctcatttaccaggagagt

SEQ ID NO: 7 - DNA, 34 bp, Artificial Sequence
  InF.HindIII-H2-214L
cggtatcgataagcttgagatggagtcagacaca

SEQ ID NO: 8 - DNA, 35 bp, Artificial Sequence
  InF.HindIII-H2-250L
cggtatcgataagcttaaaatgatgagtcctgccc

SEQ ID NO: 9 - DNA, 34 bp, Artificial Sequence
  InF.mIgCKterNotI
tctagagtcgcggccgcctaacactcattcctgt

SEQ ID NO: 10 - DNA, 1395 bp, Artificial Sequence
  H2Mab-214 Heavy chain DNA
atggacaggcttacttcctcattcctgctgctgattgtccctgcatatgtcctttcccaggttactctgaaagagtctggccctgggatattgcagccctcccagaccctcagtctgacttgttctttctctgggttttcactgagcacttctggtatgggtgtgagctggattcgtcagccttcaggaaagggtctggagtggctggcacacattttctgggatgatgacaagcgctataacccatccctgaagagccggctcacaatctccaaggatacctccagaaataaggtattcctcaagatcaccagtgtggacactgcagatactgccacatactactgtgctcgaagggtagtagctacagactggtacttcgatgtctggggcgcagggaccacggtcaccgtctcctcagccaaaacgacacccccatctgtctatccactggcccctggatctgctgcccaaactaactccatggtgaccctgggatgcctggtcaagggctatttccctgagccagtgacagtgacctggaactctggatccctgtccagcggtgtgcacaccttcccagctgtcctgcagtctgacctctacactctgagcagctcagtgactgtcccctccagcacctggcccagcgagaccgtcacctgcaacgttgcccacccggccagcagcaccaaggtggacaagaaaattgtgcccagggattgtggttgtaagccttgcatatgtacagtcccagaagtatcatctgtcttcatcttccccccaaagcccaaggatgtgctcaccattactctgactcctaaggtcacgtgtgttgtggtagacatcagcaaggatgatcccgaggtccagttcagctggtttgtagatgatgtggaggtgcacacagctcagacgcaaccccgggaggagcagttcaacagcactttccgctcagtcagtgaacttcccatcatgcaccaggactggctcaatggcaaggagttcaaatgcagggtcaacagtgcagctttccctgcccccatcgagaaaaccatctccaaaaccaaaggcagaccgaaggctccacaggtgtacaccattccacctcccaaggagcagatggccaaggataaagtcagtctgacctgcatgataacagacttcttccctgaagacattactgtggagtggcagtggaatgggcagccagcggagaactacaagaacactcagcccatcatggacacagatggctcttacttcgtctacagcaagctcaatgtgcagaagagcaactgggaggcaggaaatactttcacctgctctgtgttacatgagggcctgcacaaccaccatactgagaagagcctctcccactctcctggtaaatga

SEQ ID NO: 11 - DNA, 717 bp, Artificial Sequence
  H2Mab-214 Light chain DNA
atggagtcagacacactcctgctatgggtgctgctgctctgggttccaggctccactggtgacattgtgctcacccaatctccagcttctttggctgtgtctctaggtcagagagccaccatctcctgcagagccagtgaaagtgttgaatattatggcacaactttaatgcagtggtaccaacagaaaccaggacagccacccaaactcctcatctatgctgcatccaaagtagaatctggggtccctgccaggtttagtggcagtgggtctgggactgacttcagcctcaacatccatcctgtggaggaggatgatgttgcaatgtatttctgtcagcaaagtaggaaggttccgctcacgttcggtgctgggaccaagctggagctgaaacgggctgatgctgcaccaactgtatccatcttcccaccatccagtgagcagttaacatctggaggtgcctcagtcgtgtgcttcttgaacaacttctaccccaaagacatcaatgtcaagtggaagattgatggcagtgaacgacaaaatggcgtcctgaacagttggactgatcaggacagcaaagacagcacctacagcatgagcagcaccctcacgttgaccaaggacgagtatgaacgacataacagctatacctgtgaggccactcacaagacatcaacttcacccattgtcaagagcttcaacaggaatgagtgttag

SEQ ID NO: 12 - DNA, 1380 bp, Artificial Sequence
  H2Mab-250 Heavy chain DNA
atgaacttagggctcagcttcattttccttgccctttttttaaaaggtgtccggtgtgaggtgcagctggtggagtctgggggaggcttagtgcagccaggagggtccctgaaactctcctgtgcagcctctggattcactttcagtaactatggcatgtcttgggttcgccagactccagacaggaggctggagttggtcgcaaccattaataataatggtggtggtacctattatccagacagtgtgaagggccggttcaccatctccagagacaatgccaagaacaccctgtacctgcaaatgagcagtctgaagtctgaggacacagccatgtactactgcacaagccccggcctactatgggatgcctggggcgcagggaccacggtcaccgtctcctcagccaaaacgacacccccatctgtctatccactggcccctggatctgctgcccaaactaactccatggtgaccctgggatgcctggtcaagggctatttccctgagccagtgacagtgacctggaactctggatccctgtccagcggtgtgcacaccttcccagctgtcctgcagtctgacctctacactctgagcagctcagtgactgtcccctccagcacctggcccagcgagaccgtcacctgcaacgttgcccacccggccagcagcaccaaggtggacaagaaaattgtgcccagggattgtggttgtaagccttgcatatgtacagtcccagaagtatcatctgtcttcatcttccccccaaagcccaaggatgtgctcaccattactctgactcctaaggtcacgtgtgttgtggtagacatcagcaaggatgatcccgaggtccagttcagctggtttgtagatgatgtggaggtgcacacagctcagacgcaaccccgggaggagcagttcaacagcactttccgctcagtcagtgaacttcccatcatgcaccaggactggctcaatggcaaggagttcaaatgcagggtcaacagtgcagctttccctgcccccatcgagaaaaccatctccaaaaccaaaggcagaccgaaggctccacaggtgtacaccattccacctcccaaggagcagatggccaaggataaagtcagtctgacctgcatgataacagacttcttccctgaagacattactgtggagtggcagtggaatgggcagccagcggagaactacaagaacactcagcccatcatggacacagatggctcttacttcgtctacagcaagctcaatgtgcagaagagcaactgggaggcaggaaatactttcacctgctctgtgttacatgagggcctgcacaaccaccatactgagaagagcctctcccactctcctggtaaatga

SEQ ID NO: 13 - DNA, 720 bp, Artificial Sequence
  H2Mab-250 Light chain DNA
atgatgagtcctgcccagttcctgtttctgttagtgctctggattcgggaaaccaacggtgatgttgtgatgacccagactccactcactttgtcggtctccattggacaaccagcctccatctcttgcaagtcaagtcagagcctcttagatagtgatggaaggacatatttgaattggttgttacagaggccaggccagtctccaaagcgcctaatctatctggtgtctaaactggactctggagcccctgacaggttcactggcagtggatcagggacagattttacactgaaaatcagcagagtggaggctgaggatttgggagtttattattgctggcaaggtacacattttcctcagacgttcggtggaggcaccaagctggaaatcaaacgggctgatgctgcaccaactgtatccatcttcccaccatccagtgagcagttaacatctggaggtgcctcagtcgtgtgcttcttgaacaacttctaccccaaagacatcaatgtcaagtggaagattgatggcagtgaacgacaaaatggcgtcctgaacagttggactgatcaggacagcaaagacagcacctacagcatgagcagcaccctcacgttgaccaaggacgagtatgaacgacataacagctatacctgtgaggccactcacaagacatcaacttcacccattgtcaagagcttcaacaggaatgagtgttag

SEQ ID NO: 14 - protein, 464 aa, Artificial Sequence
  H2Mab-214 Heavy chain protein
MDRLTSSFLLLIVPAYVLSQVTLKESGPGILQPSQTLSLTCSFSGFSLSTSGMGVSWIRQPSGKGLEWLAHIFWDDDKRYNPSLKSRLTISKDTSRNKVFLKITSVDTADTATYYCARRVVATDWYFDVWGAGTTVTVSSAKTTPPSVYPLAPGSAAQTNSMVTLGCLVKGYFPEPVTVTWNSGSLSSGVHTFPAVLQSDLYTLSSSVTVPSSTWPSETVTCNVAHPASSTKVDKKIVPRDCGCKPCICTVPEVSSVFIFPPKPKDVLTITLTPKVTCVVVDISKDDPEVQFSWFVDDVEVHTAQTQPREEQFNSTFRSVSELPIMHQDWLNGKEFKCRVNSAAFPAPIEKTISKTKGRPKAPQVYTIPPPKEQMAKDKVSLTCMITDFFPEDITVEWQWNGQPAENYKNTQPIMDTDGSYFVYSKLNVQKSNWEAGNTFTCSVLHEGLHNHHTEKSLSHSPGK

SEQ ID NO: 15 - protein, 238 aa, Artificial Sequence
  H2Mab-214 Light chain protein
MESDTLLLWVLLLWVPGSTGDIVLTQSPASLAVSLGQRATISCRASESVEYYGTTLMQWYQQKPGQPPKLLIYAASKVESGVPARFSGSGSGTDFSLNIHPVEEDDVAMYFCQQSRKVPLTFGAGTKLELKRADAAPTVSIFPPSSEQLTSGGASVVCFLNNFYPKDINVKWKIDGSERQNGVLNSWTDQDSKDSTYSMSSTLTLTKDEYERHNSYTCEATHKTSTSPIVKSFNRNEC

SEQ ID NO: 16 - protein, 459 aa, Artificial Sequence
  H2Mab-250 Heavy chain protein
MNLGLSFIFLALFLKGVRCEVQLVESGGGLVQPGGSLKLSCAASGFTFSNYGMSWVRQTPDRRLELVATINNNGGGTYYPDSVKGRFTISRDNAKNTLYLQMSSLKSEDTAMYYCTSPGLLWDAWGAGTTVTVSSAKTTPPSVYPLAPGSAAQTNSMVTLGCLVKGYFPEPVTVTWNSGSLSSGVHTFPAVLQSDLYTLSSSVTVPSSTWPSETVTCNVAHPASSTKVDKKIVPRDCGCKPCICTVPEVSSVFIFPPKPKDVLTITLTPKVTCVVVDISKDDPEVQFSWFVDDVEVHTAQTQPREEQFNSTFRSVSELPIMHQDWLNGKEFKCRVNSAAFPAPIEKTISKTKGRPKAPQVYTIPPPKEQMAKDKVSLTCMITDFFPEDITVEWQWNGQPAENYKNTQPIMDTDGSYFVYSKLNVQKSNWEAGNTFTCSVLHEGLHNHHTEKSLSHSPGK

SEQ ID NO: 17 - protein, 239 aa, Artificial Sequence
  H2Mab-250 Light chain protein
MMSPAQFLFLLVLWIRETNGDVVMTQTPLTLSVSIGQPASISCKSSQSLLDSDGRTYLNWLLQRPGQSPKRLIYLVSKLDSGAPDRFTGSGSGTDFTLKISRVEAEDLGVYYCWQGTHFPQTFGGGTKLEIKRADAAPTVSIFPPSSEQLTSGGASVVCFLNNFYPKDINVKWKIDGSERQNGVLNSWTDQDSKDSTYSMSSTLTLTKDEYERHNSYTCEATHKTSTSPIVKSFNRNEC

SEQ ID NO: 18 - protein, 7 aa, Artificial Sequence
  H2Mab-214 HCDR1
TSGMGVS

SEQ ID NO: 19 - protein, 16 aa, Artificial Sequence
  H2Mab-214 HCDR2
HIFWDDDKRYNPSLKS

SEQ ID NO: 20 - protein, 11 aa, Artificial Sequence
  H2Mab-214 HCDR3
RVVATDWYFDV

SEQ ID NO: 21 - protein, 15 aa, Artificial Sequence
  H2Mab-214 LCDR1
RASESVEYYGTTLMQ

SEQ ID NO: 22 - protein, 7 aa, Artificial Sequence
  H2Mab-214 LCDR2
AASKVES

SEQ ID NO: 23 - protein, 9 aa, Artificial Sequence
  H2Mab-214 LCDR3
QQSRKVPLT

SEQ ID NO: 24 - protein, 5 aa, Artificial Sequence
  H2Mab-250 HCDR1
NYGMS

SEQ ID NO: 25 - protein, 17 aa, Artificial Sequence
  H2Mab-250 HCDR2
TINNNGGGTYYPDSVKG

SEQ ID NO: 26 - protein, 7 aa, Artificial Sequence
  H2Mab-250 HCDR3
PGLLWDA

SEQ ID NO: 27 - protein, 16 aa, Artificial Sequence
  H2Mab-250 LCDR1
KSSQSLLDSDGRTYLN

SEQ ID NO: 28 - protein, 7 aa, Artificial Sequence
  H2Mab-250 LCDR2
LVSKLDS

SEQ ID NO: 29 - protein, 9 aa, Artificial Sequence
  H2Mab-250 LCDR3
WQGTHFPQT

SEQ ID NO: 30 - protein, 53 aa, Artificial Sequence
  human HER2 600-652
CPSGVKPDLSYMPIWKFPDEEGACQPCPINCTHSCVDLDDKGCPAEQRASPLT

SEQ ID NO: 31 - protein, 20 aa, Artificial Sequence
  Human HER2 603-622
GVKPDLSYMPIWKFPDEEGA

SEQ ID NO: 32 - protein, 20 aa, Artificial Sequence
  Human HER2 613-632
IWKFPDEEGACQPCPINCTH

SEQ ID NO: 33 - protein, 10 aa, Artificial Sequence
  human HER2 613-622
IWKFPDEEGA

SEQ ID NO: 34 - protein, 8 aa, Artificial Sequence
  human HER2 611-618
MPIWKFPD

SEQ ID NO: 35 - protein, 7 aa, Artificial Sequence
  human HER2 612-618
PIWKFPD

SEQ ID NO: 36 - protein, 7 aa, Artificial Sequence
  human HER2 613-619
IWKFPDE

SEQ ID NO: 37 - protein, 20 aa, Artificial Sequence
  human HER2 p604-622C
VKPDLSYMPIWKFPDEEGAC

SEQ ID NO: 38 - protein, 20 aa, Artificial Sequence
  Linker
GGGGSGGGGSGGGGSGGGGS

SEQ ID NO: 39 - protein, 463 aa, Artificial Sequence
  H2M279 Heavy Chain Protein
MNLGLSFIFLALILKGVQCEVQLVESGGGLVQPGGSLKLSCAASGFSFSSYGIFWVRQTPDKRLELVATIKSNGGRTYYPDSVKGRFTISRDNAKNTLHLQMSSLKSEDTAMYYCAREGGDYWGQGTSVTVSSATTTAPSVYPLVPGCSDTSGSSVTLGCLVKGYFPEPVTVKWNYGALSSGVRTVSSVLQSGFYSLSSLVTVPSSTWPSQTVICNVAHPASKTELIKRIEPRIPKPSTPPGSSCPPGNILGGPSVFIFPPKPKDALMISLTPKVTCVVVDVSEDDPDVHVSWFVDNKEVHTAWTQPREAQYNSTFRVVSALPIQHQDWMRGKEFKCKVNNKALPAPIERTISKPKGRAQTPQVYTIPPPREQMSKKKVSLTCLVTNFFSEAISVEWERNGELEQDYKNTPPILDSDGTYFLYSKLTVDTDSWLQGEIFTCSVVHEALHNHHTQKNLSRSPGK

SEQ ID NO: 40 - protein, 238 aa, Artificial Sequence
  H2M279 Light Chain Protein
MGIKMETHSQVFVYMLLWLSGIEGDIVMTQSHKIMSTSVGDRVSISCKASQDVGTAVAWYQQKPGQSPILLIYWASTRHTGVPDRFTGSGSGTDFTLTISNVQSEDLADYFCQQYKSNPLTFGAGTKLELKRADAAPTVSIFPPSSEQLTSGGASVVCFLNNFYPKDINVKWKIDGSERQNGVLNSWTDQDSKDSTYSMSSTLTLTKDEYERHNSYTCEATHKTSTSPIVKSFNRNEC

SEQ ID NO: 41 - protein, 457 aa, Artificial Sequence
  H2M280 Heavy Chain Protein
MNFGLRLIFLVLTLKGVQCDVKLVESGGGLVKPGGSLKLSCAASGFTFSSYSMSWVRQTPEKRLEWVAIISSGGSYTFYPDSVKGRFTISRDNAKNTLYLQMSSLKSEDTAMYHCTREAGDYWGQGTTLTVSSAKTTPPSVYPLAPGSAAQTNSMVTLGCLVKGYFPEPVTVTWNSGSLSSGVHTFPAVLQSDLYTLSSSVTVPSSTWPSETVTCNVAHPASSTKVDKKIVPRDCGCKPCICTVPEVSSVFIFPPKPKDVLTITLTPKVTCVVVDISKDDPEVQFSWFVDDVEVHTAQTQPREEQFNSTFRSVSELPIMHQDWLNGKEFKCRVNSAAFPAPIEKTISKTKGRPKAPQVYTIPPPKEQMAKDKVSLTCMITDFFPEDITVEWQWNGQPAENYKNTQPIMDTDGSYFVYSKLNVQKSNWEAGNTFTCSVLHEGLHNHHTEKSLSHSPGK

SEQ ID NO: 42 - protein, 238 aa, Artificial Sequence
  H2M280 Light Chain Protein
MMSPAQFLFLLVLWIRETNGDIVMTQTPLTLSVTIGQPASISCKSSQSLLHSDGKTYLNWLLQRPGQSPKRLIYLVSKLDSGVPDRFTGSGSGTDFTLKISRVEADDLGIYYCWQGTHFPTFGGGTKLEIKRADAAPTVSIFPPSSEQLTSGGASVVCFLNNFYPKDINVKWKIDGSERQNGVLNSWTDQDSKDSTYSMSSTLTLTKDEYERHNSYTCEATHKTSTSPIVKSFNRNEC

SEQ ID NO: 43 - protein, 457 aa, Artificial Sequence
  H2M281 Heavy Chain Protein
MNFGLRLIFLVLTLKGVQCDVKLVESGGGLVKPGGSLKLSCAASGFTFSSYSMSWVRQTPEKRLEWVAIISSGGTYTYYTDSVKGRFTISRDDAKNTLNLQMSSLKSEDTAMFYCTREAGDYWGQGTTLTVSSAKTTPPSVYPLAPGSAAQTNSMVTLGCLVKGYFPEPVTVTWNSGSLSSGVHTFPAVLQSDLYTLSSSVTVPSSTWPSETVTCNVAHPASSTKVDKKIVPRDCGCKPCICTVPEVSSVFIFPPKPKDVLTITLTPKVTCVVVDISKDDPEVQFSWFVDDVEVHTAQTQPREEQFNSTFRSVSELPIMHQDWLNGKEFKCRVNSAAFPAPIEKTISKTKGRPKAPQVYTIPPPKEQMAKDKVSLTCMITDFFPEDITVEWQWNGQPAENYKNTQPIMDTDGSYFVYSKLNVQKSNWEAGNTFTCSVLHEGLHNHHTEKSLSHSPGK

SEQ ID NO: 44 - protein, 238 aa, Artificial Sequence
  H2M281 Light Chain Protein
MMSPAQFLFLLVLWIRETNGNVVMTQTPLTLSVTIGQPASISCKSSQSLLYSDGKTYLNWLLQRPGQSPKRLIYLVSKLDSGVPDRFTGSGSGTDFTLKISRVEAEDLGVYYCWQGTHFPTFGGGTKLEIKRADAAPTVSIFPPSSEQLTSGGASVVCFLNNFYPKDINVKWKIDGSERQNGVLNSWTDQDSKDSTYSMSSTLTLTKDEYERHNSYTCEATHKTSTSPIVKSFNRNEC

SEQ ID NO: 45 - protein, 464 aa, Artificial Sequence
  H2M282 Heavy Chain Protein
MERHWIFLLLLSVTAGVHSQVQLQQSGAELSRPGASVKMSCKAAGYTFSSYMIHWVKQRPGQGLEWIGYINPSSGYSNYNQKFKDKATLTADKSSSTAYMQLSSLTSEDSAVYYCAFYDYDGDWGQGTLVTVSAAKTTAPSVYPLAPVCGDTTGSSVTLGCLVKGYFPEPVTLTWNSGSLSSGVHTFPAVLQSDLYTLSSSVTVTSSTWPSQSITCNVAHPASSTKVDKKIEPRGPTIKPCPPCKCPAPNLLGGPSVFIFPPKIKDVLMISLSPIVTCVVVDVSEDDPDVQISWFVNNVEVHTAQTQTHREDYNSTLRVVSALPIQHQDWMSGKEFKCKVNNKDLPAPIERTISKPKGSVRAPQVYVLPPPEEEMTKKQVTLTCMVTDFMPEDIYVEWTNNGKTELNYKNTEPVLDSDGSYFMYSKLRVEKKNWVERNSYSCSVVHEGLHNHHTTKSFSRTPGK

SEQ ID NO: 46 - protein, 239 aa, Artificial Sequence
  H2M282 Light Chain Protein
MMSPAQFLFLLVLWIRDTNGDVVMTQTPLTLSVTIGQPASISCKSSQSLFHSDGRTFLNWLLQRPGQSPKRLIYKVSKLDSGVPDRFTGSGSGTDFTLKISRVEAEDLGVYYCWQGTHFPWTFGGGTKLEIKRADAAPTVSIFPPSSEQLTSGGASVVCFLNNFYPKDINVKWKIDGSERQNGVLNSWTDQDSKDSTYSMSSTLTLTKDEYERHNSYTCEATHKTSTSPIVKSFNRNEC

SEQ ID NO: 47 - protein, 459 aa, Artificial Sequence
  H2M283 Heavy Chain Protein
MNLGLSFIFLALILKGVQCEVQLVESGGGLVQPGGSLKLSCAASGFTFSSYGMSWVRQTPDKRLELVATINSNGGSTFYPDSVKGRFTISRDNAKNTLYLHMSSLKSEDTAIYYCVSPGSWFPYWGRGTLVTVSAAKTTPPSVYPLAPGSAAQTNSMVTLGCLVKGYFPEPVTVTWNSGSLSSGVHTFPAVLQSDLYTLSSSVTVPSSTWPSETVTCNVAHPASSTKVDKKIVPRDCGCKPCICTVPEVSSVFIFPPKPKDVLTITLTPKVTCVVVDISKDDPEVQFSWFVDDVEVHTAQTQPREEQFNSTFRSVSELPIMHQDWLNGKEFKCRVNSAAFPAPIEKTISKTKGRPKAPQVYTIPPPKEQMAKDKVSLTCMITDFFPEDITVEWQWNGQPAENYKNTQPIMDTDGSYFVYSKLNVQKSNWEAGNTFTCSVLHEGLHNHHTEKSLSHSPGK

SEQ ID NO: 48 - protein, 241 aa, Artificial Sequence
  H2M283 Light Chain Protein
MMSPAQFLFLLVLWIRVSETNGDVVMTQTPLTLSVTIGQPASISCKSSQSLLDSDGKTYLHWLLQRPGQSPKRLIYLVSHLDSGVPDRFTGSGSGTDFTLKISRVEAEDLGVYYCWQGTHFPQTFGGGTKLEIKRADAAPTVSIFPPSSEQLTSGGASVVCFLNNFYPKDINVKWKIDGSERQNGVLNSWTDQDSKDSTYSMSSTLTLTKDEYERHNSYTCEATHKTSTSPIVKSFNRNEC

SEQ ID NO: 49 - protein, 462 aa, Artificial Sequence
  H2M284 Heavy Chain Protein
MGRLTSSFLLLIVPAYVLSQVTLKESGPGILQPSQTLSLTCSFSGFSLSTSGVGVGWIRQPSGKGLEWLAHIWWDDDKNYNPALKSRLTISKDTSTNQGFLKIASVDTADTATYFCARIEGQKGFAYWGQGTLVTVSAAKTTPPSVYPLAPGSAAQTNSMVTLGCLVKGYFPEPVTVTWNSGSLSSGVHTFPAVLQSDLYTLSSSVTVPSSTWPSETVTCNVAHPASSTKVDKKIVPRDCGCKPCICTVPEVSSVFIFPPKPKDVLTITLTPKVTCVVVDISKDDPEVQFSWFVDDVEVHTAQTQPREEQFNSTFRSVSELPIMHQDWLNGKEFKCRVNSAAFPAPIEKTISKTKGRPKAPQVYTIPPPKEQMAKDKVSLTCMITDFFPEDITVEWQWNGQPAENYKNTQPIMDTDGSYFVYSKLNVQKSNWEAGNTFTCSVLHEGLHNHHTEKSLSHSPGK

SEQ ID NO: 50 - protein, 240 aa, Artificial Sequence
  H2M284 Light Chain Protein
MDSQAQVLMLLLLWVSGTCGDIVMSQSPSSLAVSVGEKVTMSCKSSQSLLYSRNQKNYLAWYQQKPGQSPKLLIYWASTRESGVPDRFTGSGSGTDFTLTISSVKAEDLAVYYCQQYYSSPYTFGGGTKLEIKRADAAPTVSIFPPSSEQLTSGGASVVCFLNNFYPKDINVKWKIDGSERQNGVLNSWTDQDSKDSTYSMSSTLTLTKDEYERHNSYTCEATHKTSTSPIVKSFNRNEC

SEQ ID NO: 51 - protein, 463 aa, Artificial Sequence
  H2M285 Heavy Chain Protein
MNLGLSFIFLVLILKGVQCEVQLVESGGGLVQPGGSLKLSCAASGFTFSNYGIFWVRQTPDKRLELVATVKSNGGSTYYPDSVKGRFTISRDNAKKTLYLQMSSLKSEDTAMYYCAREGGDYWGQGTSVTVSSATTTAPSVYPLVPGCSDTSGSSVTLGCLVKGYFPEPVTVKWNYGALSSGVRTVSSVLQSGFYSLSSLVTVPSSTWPSQTVICNVAHPASKTELIKRIEPRIPKPSTPPGSSCPPGNILGGPSVFIFPPKPKDALMISLTPKVTCVVVDVSEDDPDVHVSWFVDNKEVHTAWTQPREAQYNSTFRVVSALPIQHQDWMRGKEFKCKVNNKALPAPIERTISKPKGRAQTPQVYTIPPPREQMSKKKVSLTCLVTNFFSEAISVEWERNGELEQDYKNTPPILDSDGTYFLYSKLTVDTDSWLQGEIFTCSVVHEALHNHHTQKNLSRSPGK

SEQ ID NO: 52 - protein, 238 aa, Artificial Sequence
  H2M285 Light Chain Protein
MGIKMETHSQVFVYMLLWLSGVEGDIVMTQSHKFMSTSVGDRVSITCKASQDVGTAVAWYQQKPGQSPKLLIYWTSTRHTGVPDRFTGSGSGTDFTLTIRNVQSEDLADYFCQQYNRNPLTFGAGTRLELKRADAAPTVSIFPPSSEQLTSGGASVVCFLNNFYPKDINVKWKIDGSERQNGVLNSWTDQDSKDSTYSMSSTLTLTKDEYERHNSYTCEATHKTSTSPIVKSFNRNEC

SEQ ID NO: 53 - protein, 455 aa, Artificial Sequence
  H2M286 Heavy Chain Protein
MRVLILLWLFTAFPGILSDVQLQESGPGLVKPSQSLSLTCTVTGYSITSDYGWNWIRQFPGNKLEWMGYIRYSGITSYNPSLKSRISITRDTSKNQFFLQLNSVTTEDTATYYCTREVLSWGQGTTLTVSSAKTTPPSVYPLAPGSAAQTNSMVTLGCLVKGYFPEPVTVTWNSGSLSSGVHTFPAVLQSDLYTLSSSVTVPSSTWPSETVTCNVAHPASSTKVDKKIVPRDCGCKPCICTVPEVSSVFIFPPKPKDVLTITLTPKVTCVVVDISKDDPEVQFSWFVDDVEVHTAQTQPREEQFNSTFRSVSELPIMHQDWLNGKEFKCRVNSAAFPAPIEKTISKTKGRPKAPQVYTIPPPKEQMAKDKVSLTCMITDFFPEDITVEWQWNGQPAENYKNTQPIMDTDGSYFVYSKLNVQKSNWEAGNTFTCSVLHEGLHNHHTEKSLSHSPGK

SEQ ID NO: 54 - protein, 238 aa, Artificial Sequence
  H2M286 Light Chain Protein
MKLPVRLLVLMFWIPASSSDVVMTQTPLSLPVSLGDQASISCRSSQSLVHSNGNTYLHWFLQKPGQSPKLLIYKVSNRFSGVPARFSGSGSGTDFTLKISRVEAEDLGVYFCSQSTHVPPTFGGGTKLEIKRADAAPTVSIFPPSSEQLTSGGASVVCFLNNFYPKDINVKWKIDGSERQNGVLNSWTDQDSKDSTYSMSSTLTLTKDEYERHNSYTCEATHKTSTSPIVKSFNRNEC

SEQ ID NO: 55 - protein, 457 aa, Artificial Sequence
  H2M287 Heavy Chain Protein
MNFGLRLIFLVLTLKGVQCDVKLVESGGGLVKPGGSLKLSCAASGFTFSSYSMSWVRQTPEKRLEWVAIISSGGSYIFYPDSVKGRFTISRDNAKNTLYLQMSSLKSEDTAMYYCTREAGDYWGQGTTLTVSSAKTTPPSVYPLAPGSAAQTNSMVTLGCLVKGYFPEPVTVTWNSGSLSSGVHTFPAVLQSDLYTLSSSVTVPSSTWPSETVTCNVAHPASSTKVDKKIVPRDCGCKPCICTVPEVSSVFIFPPKPKDVLTITLTPKVTCVVVDISKDDPEVQFSWFVDDVEVHTAQTQPREEQFNSTFRSVSELPIMHQDWLNGKEFKCRVNSAAFPAPIEKTISKTKGRPKAPQVYTIPPPKEQMAKDKVSLTCMITDFFPEDITVEWQWNGQPAENYKNTQPIMDTDGSYFVYSKLNVQKSNWEAGNTFTCSVLHEGLHNHHTEKSLSHSPGK

SEQ ID NO: 56 - protein, 238 aa, Artificial Sequence
  H2M287 Light Chain Protein
MMSPAQFLFLLVLWIRETNGDVVMTQTPLTLSVTIGQPASISCKSSQSLLHSDGKTYLNWLLQRPGQSPKRLIYLVSKLDSGVPDRFTGSGSGTDFTLKISRVEAEDLGVYYCWQGTHFPTFGGGTKLEIKRADAAPTVSIFPPSSEQLTSGGASVVCFLNNFYPKDINVKWKIDGSERQNGVLNSWTDQDSKDSTYSMSSTLTLTKDEYERHNSYTCEATHKTSTSPIVKSFNRNEC

SEQ ID NO: 57 - protein, 457 aa, Artificial Sequence
  H2M288 Heavy Chain Protein
MNFGLRLIFLVLTLKGVQCDVKLVESGGGLVKPGGSLKLSCAASGFTFSRYSLSWVRQTPEKRLEWVAVISSGGRYTFYPDGVKGRFTISRDDAKNTLYLQMSSLRSEDTAMYFCTREAGDYWGQGTPLTVSSAKTTPPSVYPLAPGSAAQTNSMVTLGCLVKGYFPEPVTVTWNSGSLSSGVHTFPAVLQSDLYTLSSSVTVPSSTWPSETVTCNVAHPASSTKVDKKIVPRDCGCKPCICTVPEVSSVFIFPPKPKDVLTITLTPKVTCVVVDISKDDPEVQFSWFVDDVEVHTAQTQPREEQFNSTFRSVSELPIMHQDWLNGKEFKCRVNSAAFPAPIEKTISKTKGRPKAPQVYTIPPPKEQMAKDKVSLTCMITDFFPEDITVEWQWNGQPAENYKNTQPIMDTDGSYFVYSKLNVQKSNWEAGNTFTCSVLHEGLHNHHTEKSLSHSPGK

SEQ ID NO: 58 - protein, 238 aa, Artificial Sequence; identical to SEQ ID NO: 56
  H2M288 Light Chain Protein

SEQ ID NO: 59 - protein, 464 aa, Artificial Sequence
  H2M289 Heavy Chain Protein
MGWSWIFLSLLSVTAGVFSEVQLQQSGPELVKPGASVKISCKASGYSFTGFFMNWVMQSHGKSLEWIGRINPYNGDTFYNQKFNDKATLTVDKSSRTAHMDLRNLASEDSAVYYCATISGNYRGYAMDNWGQGTSVTVSSAKTTPPSVYPLAPGSAAQTNSMVTLGCLVKGYFPEPVTVTWNSGSLSSGVHTFPAVLQSDLYTLSSSVTVPSSTWPSETVTCNVAHPASSTKVDKKIVPRDCGCKPCICTVPEVSSVFIFPPKPKDVLTITLTPKVTCVVVDISKDDPEVQFSWFVDDVEVHTAQTQPREEQFNSTFRSVSELPIMHQDWLNGKEFKCRVNSAAFPAPIEKTISKTKGRPKAPQVYTIPPPKEQMAKDKVSLTCMITDFFPEDITVEWQWNGQPAENYKNTQPIMDTDGSYFVYSKLNVQKSNWEAGNTFTCSVLHEGLHNHHTEKSLSHSPGK

SEQ ID NO: 60 - protein, 238 aa, Artificial Sequence
  H2M289 Light Chain Protein
MKLPVRLLVLMFWIPASSSDVLMTQTPLSLPVSLGDQASISCRSSQTILHTNGNTYLEWYLQKPGQSPKLLIYKVSNRFSGVPDRFSGSGSGTDFTLKISRVEAEDLGVYYCFQGSRVPPTFGGGTKLEIKRADAAPTVSIFPPSSEQLTSGGASVVCFLNNFYPKDINVKWKIDGSERQNGVLNSWTDQDSKDSTYSMSSTLTLTKDEYERHNSYTCEATHKTSTSPIVKSFNRNEC

SEQ ID NO: 61 - protein, 457 aa, Artificial Sequence; identical to SEQ ID NO: 55
  H2M290 Heavy Chain Protein

SEQ ID NO: 62 - protein, 238 aa, Artificial Sequence
  H2M290 Light Chain Protein
MMSPAQFLFLLVLWIRETNGDVVMTQTPLTLSVTIGQPASISCKSSQSLLHSDGKTYLNWLLQRPGQSPKRLLYLVSNLDSGVPDRFTGSGSGTDFTLKISRVEAEDLGIYYCWQGTHFPTFGGGTKLEIKRADAAPTVSIFPPSSEQLTSGGASVVCFLNNFYPKDINVKWKIDGSERQNGVLNSWTDQDSKDSTYSMSSTLTLTKDEYERHNSYTCEATHKTSTSPIVKSFNRNEC

SEQ ID NO: 63 - protein, 463 aa, Artificial Sequence
  H2M291 Heavy Chain Protein
MGWSWIFLFLLSGTAGVHSEVQLQQSGPELVKPGASMKISCKASGYSFTGYTMNWVKQSHGKNLEWIGLINPYNGNTRYNQKFQDKATLTVDRSSSTAYMELLSLTSEDSAVYYCVKEPSDYWGQGTTLTVSSATTTAPSVYPLVPGCSDTSGSSVTLGCLVKGYFPEPVTVKWNYGALSSGVRTVSSVLQSGFYSLSSLVTVPSSTWPSQTVICNVAHPASKTELIKRIEPRIPKPSTPPGSSCPPGNILGGPSVFIFPPKPKDALMISLTPKVTCVVVDVSEDDPDVHVSWFVDNKEVHTAWTQPREAQYNSTFRVVSALPIQHQDWMRGKEFKCKVNNKALPAPIERTISKPKGRAQTPQVYTIPPPREQMSKKKVSLTCLVTNFFSEAISVEWERNGELEQDYKNTPPILDSDGTYFLYSKLTVDTDSWLQGEIFTCSVVHEALHNHHTQKNLSRSPGK

SEQ ID NO: 64 - protein, 238 aa, Artificial Sequence
  H2M291 Light Chain Protein
MKLPVRLLVLMFWIPASSSDVVMTQTPLSLPVSLGDQASISCRSSQSLVHINGNTYLHWYLQKPGQSPKLLIYKVSKRFSGVPDRFSGSGSGTDFTLKISRVEAADLGVYFCSQSTHVPPTFGGGTKLEIKRADAAPTVSIFPPSSEQLTSGGASVVCFLNNFYPKDINVKWKIDGSERQNGVLNSWTDQDSKDSTYSMSSTLTLTKDEYERHNSYTCEATHKTSTSPIVKSFNRNEC

SEQ ID NO: 65 - protein, 463 aa, Artificial Sequence
  H2M292 Heavy Chain Protein
MGWSWIFLFLLSGTAGVHSEVQLQQSGPELVKPGASRKISCKASGYSFTGYTMNWVKKSHGKNLEWIGLINPSNGGTRYNQKFKDKATLTVDKSSSTAYMELLSLTSEDSAVYYCVKEPSDYWGQGTTLTVSSATTTAPSVYPLVPGCSDTSGSSVTLGCLVKGYFPEPVTVKWNYGALSSGVRTVSSVLQSGFYSLSSLVTVPSSTWPSQTVICNVAHPASKTELIKRIEPRIPKPSTPPGSSCPPGNILGGPSVFIFPPKPKDALMISLTPKVTCVVVDVSEDDPDVHVSWFVDNKEVHTAWTQPREAQYNSTFRVVSALPIQHQDWMRGKEFKCKVNNKALPAPIERTISKPKGRAQTPQVYTIPPPREQMSKKKVSLTCLVTNFFSEAISVEWERNGELEQDYKNTPPILDSDGTYFLYSKLTVDTDSWLQGEIFTCSVVHEALHNHHTQKNLSRSPGK

SEQ ID NO: 66 - protein, 238 aa, Artificial Sequence
  H2M292 Light Chain Protein
MKLPVRLLVLMFWIPASSSDVVMTQTPLSLPVSLGDQASISCRSSQSLVHSNGNTYLHWYLQKPGQSPKLLIYKVSNRFSGVPDRFSGRGSGTDFTLKISRVEAEDLGIYFCSQSTHVPPTFGGGTKLEIKRADAAPTVSIFPPSSEQLTSGGASVVCFLNNFYPKDINVKWKIDGSERQNGVLNSWTDQDSKDSTYSMSSTLTLTKDEYERHNSYTCEATHKTSTSPIVKSFNRNEC

SEQ ID NO: 67 - protein, 463 aa, Artificial Sequence
  H2M293 Heavy Chain Protein
MNLGLSFIFLALILKGVQCEVQLVESGGGLVQPGGSLKLSCAASGFTFSNYGIFWVRQTPDKRLELVATVKSNGGSTYYPDSVKGRFTISRDNAKKTLYLQMSSLKSEDTAMYYCAREGGDYWGQGTSVTVSSATTTAPSVYPLVPGCSDTSGSSVTLGCLVKGYFPEPVTVKWNYGALSSGVRTVSSVLQSGFYSLSSLVTVPSSTWPSQTVICNVAHPASKTELIKRIEPRIPKPSTPPGSSCPPGNILGGPSVFIFPPKPKDALMISLTPKVTCVVVDVSEDDPDVHVSWFVDNKEVHTAWTQPREAQYNSTFRVVSALPIQHQDWMRGKEFKCKVNNKALPAPIERTISKPKGRAQTPQVYTIPPPREQMSKKKVSLTCLVTNFFSEAISVEWERNGELEQDYKNTPPILDSDGTYFLYSKLTVDTDSWLQGEIFTCSVVHEALHNHHTQKNLSRSPGK

SEQ ID NO: 68 - protein, 238 aa, Artificial Sequence
  H2M293 Light Chain Protein
MGIKMETHSQVFVYMLLWLSGVEGDIVMTQSHKFMSTSVGDRVSITCKASQDVGTAVAWYQQKPGQSPKLLIYWTSTRHIGVPDRFTGSGSGTDFTLTIRNVQSEDLANYFCQQYSKNPLTFGAGTKLELKRADAAPTVSIFPPSSEQLTSGGASVVCFLNNFYPKDINVKWKIDGSERQNGVLNSWTDQDSKDSTYSMSSTLTLTKDEYERHNSYTCEATHKTSTSPIVKSFNRNEC

SEQ ID NO: 69 - protein, 468 aa, Artificial Sequence
  H2M294 Heavy Chain Protein
MSTEHRPLSVNLGLSFIFLALILKGVQCEVQLVESGGGLVQPGGSLKLSCAASGFTFSSYGMSWVRQTPDKRLELVATINSNGGGTYYPDSVKGRFTISRDNAKNTLYLQMSSLKSEDTAIYYCASPGSWFPYWGQGTLVTVSAAKTTPPSVYPLAPGSAAQTNSMVTLGCLVKGYFPEPVTVTWNSGSLSSGVHTFPAVLQSDLYTLSSSVTVPSSTWPSETVTCNVAHPASSTKVDKKIVPRDCGCKPCICTVPEVSSVFIFPPKPKDVLTITLTPKVTCVVVDISKDDPEVQFSWFVDDVEVHTAQTQPREEQFNSTFRSVSELPIMHQDWLNGKEFKCRVNSAAFPAPIEKTISKTKGRPKAPQVYTIPPPKEQMAKDKVSLTCMITDFFPEDITVEWQWNGQPAENYKNTQPIMDTDGSYFVYSKLNVQKSNWEAGNTFTCSVLHEGLHNHHTEKSLSHSPGK

SEQ ID NO: 70 - protein, 239 aa, Artificial Sequence
  H2M294 Light Chain Protein
MMSPAQFLFLLVLWIRETNGDVVMTQTPLTLSVTIGQPASISCKSSQSLLDSDGKTYLHWLLQRPGQSPRRLIFLVSKLDSGVPDRFTGSGSGTDFTLKISRVEAEDLGVYYCWQGTHFPQTFGGGTKLEIKRADAAPTVSIFPPSSEQLTSGGASVVCFLNNFYPKDINVKWKIDGSERQNGVLNSWTDQDSKDSTYSMSSTLTLTKDEYERHNSYTCEATHKTSTSPIVKSFNRNEC

SEQ ID NO: 71 - protein, 457 aa, Artificial Sequence
  H2M295 Heavy Chain Protein
MGWSWIFLFLLSGTAGVHSEVQLQQSGPELVKPGASRKISCKASGYSFTGYTMNWVKKSHGKNLEWIGLINPYNGGTRYNQKFKGKATLTVDKSSSTAYMELLSLTSEDSAVYYCVKEPSDYWGQGTTLTVSSAKTTPPSVYPLAPGSAAQTNSMVTLGCLVKGYFPEPVTVTWNSGSLSSGVHTFPAVLQSDLYTLSSSVTVPSSTWPSETVTCNVAHPASSTKVDKKIVPRDCGCKPCICTVPEVSSVFIFPPKPKDVLTITLTPKVTCVVVDISKDDPEVQFSWFVDDVEVHTAQTQPREEQFNSTFRSVSELPIMHQDWLNGKEFKCRVNSAAFPAPIEKTISKTKGRPKAPQVYTIPPPKEQMAKDKVSLTCMITDFFPEDITVEWQWNGQPAENYKNTQPIMDTDGSYFVYSKLNVQKSNWEAGNTFTCSVLHEGLHNHHTEKSLSHSPGK

SEQ ID NO: 72 - protein, 238 aa, Artificial Sequence
  H2M295 Light Chain Protein
MKLPVRLLVLMFWIPASSSDVVMTQTPLSLPVSLGDQASISCRSSQSLVHSNGNTYLHWYLQKPGQSPKLLIYKVSKRFSGVPDRFSGCGSGTDFTLKISRLEAEDLGVYFCSQSSHVPPTFGGGTKLEIKRADAAPTVSIFPPSSEQLTSGGASVVCFLNNFYPKDINVKWKIDGSERQNGVLNSWTDQDSKDSTYSMSSTLTLTKDEYERHNSYTCEATHKTSTSPIVKSFNRNEC

SEQ ID NO: 73 - protein, 462 aa, Artificial Sequence
  H2M296 Heavy Chain Protein
MGRLTSSFLLLIVPAYVLSQVTLKESGPGILQPSQTLSLTCSFSGFSLSTSGMGVGWIRQPSGKGLEWLAHIWWDDDKRYNPALKSRLTISKDTSSNQVFLKIANVDTSDTATYYCSRIEGQRGFAYWGQGTLVTVSAAKTTPPSVYPLAPGSAAQTNSMVTLGCLVKGYFPEPVTVTWNSGSLSSGVHTFPAVLQSDLYTLSSSVTVPSSTWPSETVTCNVAHPASSTKVDKKIVPRDCGCKPCICTVPEVSSVFIFPPKPKDVLTITLTPKVTCVVVDISKDDPEVQFSWFVDDVEVHTAQTQPREEQFNSTFRSVSELPIMHQDWLNGKEFKCRVNSAAFPAPIEKTISKTKGRPKAPQVYTIPPPKEQMAKDKVSLTCMITDFFPEDITVEWQWNGQPAENYKNTQPIMDTDGSYFVYSKLNVQKSNWEAGNTFTCSVLHEGLHNHHTEKSLSHSPGK

SEQ ID NO: 74 - protein, 240 aa, Artificial Sequence
  H2M296 Light Chain Protein
MDSQAQVLMLLLLWVSGTCGDIVMSQSPSSLAVSVGEMITMTCKSSQSLLYSRNQKNYLAWYQQKPGQSPKLLIYWASTRESGVPDRFTGSGSGTDFTLTISSVKAEDLAVYYCQQYYSQPYTFGGGTKLEIKRADAAPTVSIFPPSSEQLTSGGASVVCFLNNFYPKDINVKWKIDGSERQNGVLNSWTDQDSKDSTYSMSSTLTLTKDEYERHNSYTCEATHKTSTSPIVKSFNRNEC

SEQ ID NO: 75 - protein, 463 aa, Artificial Sequence; identical to SEQ ID NO: 39
  H2M297 Heavy Chain Protein

SEQ ID NO: 76 - protein, 238 aa, Artificial Sequence
  H2M297 Light Chain Protein
MKLPVRLLVLMFWIPASSSDVLMTQTPLSLPVSLGDQASISCRSSQSVVHSNGNTYLEWYLQKPGQSPKLLIYKVSNRFSGVPDRFSGSGSGTDFTLKISRVEAEDLGIYYCFQGSRVPPTFGGGTKLEIKRADAAPTVSIFPPSSEQLTSGGASVVCFLNNFYPKDINVKWKIDGSERQNGVLNSWTDQDSKDSTYSMSSTLTLTKDEYERHNNYTCEATHKTSTSPIVKSFNRNEC

SEQ ID NO: 77 - protein, 457 aa, Artificial Sequence
  H2M298 Heavy Chain Protein
MNFGLRLIFLVLTLKGVQCDVKLVESGGGLVKPGGSLKLSCAASGFTFSRYSMSWVRQTPEKKLEWVAIISTGGSYMFYPDSAKGRFTISRDDAKNTLYLQMSSLKSEDTAMYYCTREAGDYWGQGTTLTVSSAKTTPPSVYPLAPGSAAQTNSMVTLGCLVKGYFPEPVTVTWNSGSLSSGVHTFPAVLQSDLYTLSSSVTVPSSTWPSETVTCNVAHPASSTKVDKKIVPRDCGCKPCICTVPEVSSVFIFPPKPKDVLTITLTPKVTCVVVDISKDDPEVQFSWFVDDVEVHTAQTQPREEQFNSTFRSVSELPIMHQDWLNGKEFKCRVNSAAFPAPIEKTISKTKGRPKAPQVYTIPPPKEQMAKDKVSLTCMITDFFPEDITVEWQWNGQPAENYKNTQPIMDTDGSYFVYSKLNVQKSNWEAGNTFTCSVLHEGLHNHHTEKSLSHSPGK

SEQ ID NO: 78 - protein, 238 aa, Artificial Sequence
  H2M298 Light Chain Protein
MMSPAQFLFLLVLWIRETNGDVVMTQTPLTLSVTIGQPASISCKSSQSLLHSDGKTYLNWLLQRPGQSPRRLIYLVSKLDSGVPDRFTGSGSGTDFTLKISRVESEDLGVYYCWQGTHFPTFGGGTKLEIKRADAAPTVSIFPPSSEQLTSGGASVVCFLNNFYPKDINVKWKIDGSERQNGVLNSWTDQDSKDSTYSMSSTLTLTKDEYERHNSYTCEATHKTSTSPIVKSFNRNEC

SEQ ID NO: 79 - protein, 457 aa, Artificial Sequence
  H2M299 Heavy Chain Protein
MNLGLSFIFLALILKGVQCEVQLVESGGGLVQPGGSLKLSCAASGFTFNIYGIFWVRQTPDKRLELVATIHSNGGRIYYPDSVKGRFTISRDNAKNTLYLQMSSLKSEDTAMYYCAREGGDYWGQGTSVTVSSAKTTPPSVYPLAPGSAAQTNSMVTLGCLVKGYFPEPVTVTWNSGSLSSGVHTFPAVLQSDLYTLSSSVTVPSSTWPSETVTCNVAHPASSTKVDKKIVPRDCGCKPCICTVPEVSSVFIFPPKPKDVLTITLTPKVTCVVVDISKDDPEVQFSWFVDDVEVHTAQTQPREEQFNSTFRSVSELPIMHQDWLNGKEFKCRVNSAAFPAPIEKTISKTKGRPKAPQVYTIPPPKEQMAKDKVSLTCMITDFFPEDITVEWQWNGQPAENYKNTQPIMDTDGSYFVYSKLNVQKSNWEAGNTFTCSVLHEGLHNHHTEKSLSHSPGK

SEQ ID NO: 80 - protein, 238 aa, Artificial Sequence
  H2M299 Light Chain Protein
MGIKMETHSQVFVYMLLWLSGVEGDIVMTQSHKVMATSVGDRVSITCKASQDVGTAVAWYQQKPGQSPKLLIYWASTRHTGVPDRFTGSGSGTDFTLTINNVLSEDLVDYFCQQYRRYPLTFGAGTKLELKRADAAPTVSIFPPSSEQLTSGGASVVCFLNNFYPKDINVKWKIDGSERQNGVLNSWTDQDSKDSTYSMSSTLTLTKDEYERHNSYTCEATHKTSTSPIVKSFNRNEC

SEQ ID NO: 81 - protein, 5 aa, Artificial Sequence
  H2M279H-CDR1
SYGIF

SEQ ID NO: 82 - protein, 17 aa, Artificial Sequence
  H2M279H-CDR2
TIKSNGGRTYYPDSVKG

SEQ ID NO: 83 - protein, 5 aa, Artificial Sequence
  H2M279H-CDR3
EGGDY

SEQ ID NO: 84 - protein, 11 aa, Artificial Sequence
  H2M279L-CDR1
KASQDVGTAVA

SEQ ID NO: 85 - protein, 7 aa, Artificial Sequence
  H2M279L-CDR2
WASTRHT

SEQ ID NO: 86 - protein, 9 aa, Artificial Sequence
  H2M279L-CDR3
QQYKSNPLT

SEQ ID NO: 87 - protein, 5 aa, Artificial Sequence
  H2M280H-CDR1
SYSMS

SEQ ID NO: 88 - protein, 17 aa, Artificial Sequence
  H2M280H-CDR2
IISSGGSYTFYPDSVKG

SEQ ID NO: 89 - protein, 5 aa, Artificial Sequence
  H2M280H-CDR3
EAGDY

SEQ ID NO: 90 - protein, 16 aa, Artificial Sequence
  H2M280L-CDR1
KSSQSLLHSDGKTYLN

SEQ ID NO: 91 - protein, 7 aa, Artificial Sequence
  H2M280L-CDR2
LVSKLDS

SEQ ID NO: 92 - protein, 8 aa, Artificial Sequence
  H2M280L-CDR3
WQGTHFPT

SEQ ID NO: 93 - protein, 5 aa, Artificial Sequence
  H2M281H-CDR1
SYSMS

SEQ ID NO: 94 - protein, 17 aa, Artificial Sequence
  H2M281H-CDR2
IISSGGTYTYYTDSVKG

SEQ ID NO: 95 - protein, 5 aa, Artificial Sequence
  H2M281H-CDR3
EAGDY

SEQ ID NO: 96 - protein, 16 aa, Artificial Sequence
  H2M281L-CDR1
KSSQSLLYSDGKTYLN

SEQ ID NO: 97 - protein, 7 aa, Artificial Sequence
  H2M281L-CDR2
LVSKLDS

SEQ ID NO: 98 - protein, 8 aa, Artificial Sequence
  H2M281L-CDR3
WQGTHFPT

SEQ ID NO: 99 - protein, 5 aa, Artificial Sequence
  H2M282H-CDR1
SYMIH

SEQ ID NO: 100 - protein, 17 aa, Artificial Sequence
  H2M282H-CDR2
YINPSSGYSNYNQKFKD

SEQ ID NO: 101 - protein, 6 aa, Artificial Sequence
  H2M282H-CDR3
YDYDGD

SEQ ID NO: 102 - protein, 16 aa, Artificial Sequence
  H2M282L-CDR1
KSSQSLFHSDGRTFLN

SEQ ID NO: 103 - protein, 7 aa, Artificial Sequence
  H2M282L-CDR2
KVSKLDS

SEQ ID NO: 104 - protein, 9 aa, Artificial Sequence
  H2M282L-CDR3
WQGTHFPWT

SEQ ID NO: 105 - protein, 5 aa, Artificial Sequence
  H2M283H-CDR1
SYGMS

SEQ ID NO: 106 - protein, 17 aa, Artificial Sequence
  H2M283H-CDR2
TINSNGGSTFYPDSVKG

SEQ ID NO: 107 - protein, 7 aa, Artificial Sequence
  H2M283H-CDR3
PGSWFPY

SEQ ID NO: 108 - protein, 16 aa, Artificial Sequence
  H2M283L-CDR1
KSSQSLLDSDGKTYLH

SEQ ID NO: 109 - protein, 7 aa, Artificial Sequence
  H2M283L-CDR2
LVSHLDS

SEQ ID NO: 110 - protein, 9 aa, Artificial Sequence
  H2M283L-CDR3
WQGTHFPQT

SEQ ID NO: 111 - protein, 7 aa, Artificial Sequence
  H2M284H-CDR1
TSGVGVG

SEQ ID NO: 112 - protein, 16 aa, Artificial Sequence
  H2M284H-CDR2
HIWWDDDKNYNPALKS

SEQ ID NO: 113 - protein, 9 aa, Artificial Sequence
  H2M284H-CDR3
IEGQKGFAY

SEQ ID NO: 114 - protein, 17 aa, Artificial Sequence
  H2M284L-CDR1
KSSQSLLYSRNQKNYLA

SEQ ID NO: 115 - protein, 7 aa, Artificial Sequence
  H2M284L-CDR2
WASTRES

SEQ ID NO: 116 - protein, 9 aa, Artificial Sequence
  H2M284L-CDR3
QQYYSSPYT

SEQ ID NO: 117 - protein, 5 aa, Artificial Sequence
  H2M285H-CDR1
NYGIF

SEQ ID NO: 118 - protein, 17 aa, Artificial Sequence
  H2M285H-CDR2
TVKSNGGSTYYPDSVKG

SEQ ID NO: 119 - protein, 5 aa, Artificial Sequence
  H2M285H-CDR3
EGGDY

SEQ ID NO: 120 - protein, 11 aa, Artificial Sequence
  H2M285L-CDR1
KASQDVGTAVA

SEQ ID NO: 121 - protein, 7 aa, Artificial Sequence
  H2M285L-CDR2
WTSTRHT

SEQ ID NO: 122 - protein, 9 aa, Artificial Sequence
  H2M285L-CDR3
QQYNRNPLT

SEQ ID NO: 123 - protein, 6 aa, Artificial Sequence
  H2M286H-CDR1
  MISC_FEATURE (1)..(5): CDR1 has not yet determined
  MISC_FEATURE (1)..(5): CDR1 has not yet determined.  The length of this sequence does not mean the length of actual CDR1.
  misc_feature (6)..(6): Xaa can be any naturally occurring amino acid
XXXXXX

SEQ ID NO: 124 - protein, 10 aa, Artificial Sequence
  H2M286H-CDR2
  MISC_FEATURE (1)..(10): CDR2 has not yet determined.  The length of this sequence does not mean the length of actual CDR2.
XXXXXXXXXX

SEQ ID NO: 125 - protein, 5 aa, Artificial Sequence
  H2M286H-CDR3
  MISC_FEATURE (1)..(5): CDR3 has not yet determined.  The length of this sequence does not mean the length of actual CDR3.
XXXXX

SEQ ID NO: 126 - protein, 16 aa, Artificial Sequence
  H2M286L-CDR1
RSSQSLVHSNGNTYLH

SEQ ID NO: 127 - protein, 7 aa, Artificial Sequence
  H2M286L-CDR2
KVSNRFS

SEQ ID NO: 128 - protein, 9 aa, Artificial Sequence
  H2M286L-CDR3
SQSTHVPPT

SEQ ID NO: 129 - protein, 5 aa, Artificial Sequence
  H2M287H-CDR1
SYSMS

SEQ ID NO: 130 - protein, 17 aa, Artificial Sequence
  H2M287H-CDR2
IISSGGSYIFYPDSVKG

SEQ ID NO: 131 - protein, 5 aa, Artificial Sequence
  H2M287H-CDR3
EAGDY

SEQ ID NO: 132 - protein, 16 aa, Artificial Sequence
  H2M287L-CDR1
KSSQSLLHSDGKTYLN

SEQ ID NO: 133 - protein, 7 aa, Artificial Sequence
  H2M287L-CDR2
LVSKLDS

SEQ ID NO: 134 - protein, 8 aa, Artificial Sequence
  H2M287L-CDR3
WQGTHFPT

SEQ ID NO: 135 - protein, 5 aa, Artificial Sequence
  H2M288H-CDR1
RYSLS

SEQ ID NO: 136 - protein, 17 aa, Artificial Sequence
  H2M288H-CDR2
VISSGGRYTFYPDGVKG

SEQ ID NO: 137 - protein, 5 aa, Artificial Sequence
  H2M288H-CDR3
EAGDY

SEQ ID NO: 138 - protein, 16 aa, Artificial Sequence
  H2M288L-CDR1
KSSQSLLHSDGKTYLN

SEQ ID NO: 139 - protein, 7 aa, Artificial Sequence
  H2M288L-CDR2
LVSKLDS

SEQ ID NO: 140 - protein, 8 aa, Artificial Sequence
  H2M288L-CDR3
WQGTHFPT

SEQ ID NO: 141 - protein, 5 aa, Artificial Sequence
  H2M289H-CDR1
GFFMN

SEQ ID NO: 142 - protein, 17 aa, Artificial Sequence
  H2M289H-CDR2
RINPYNGDTFYNQKFND

SEQ ID NO: 143 - protein, 12 aa, Artificial Sequence
  H2M289H-CDR3
ISGNYRGYAMDN

SEQ ID NO: 144 - protein, 16 aa, Artificial Sequence
  H2M289L-CDR1
RSSQTILHTNGNTYLE

SEQ ID NO: 145 - protein, 7 aa, Artificial Sequence
  H2M289L-CDR2
KVSNRFS

SEQ ID NO: 146 - protein, 9 aa, Artificial Sequence
  H2M289L-CDR3
FQGSRVPPT

SEQ ID NO: 147 - protein, 5 aa, Artificial Sequence
  H2M290H-CDR1
SYSMS

SEQ ID NO: 148 - protein, 17 aa, Artificial Sequence
  H2M290H-CDR2
IISSGGSYIFYPDSVKG

SEQ ID NO: 149 - protein, 5 aa, Artificial Sequence
  H2M290H-CDR3
EAGDY

SEQ ID NO: 150 - protein, 16 aa, Artificial Sequence
  H2M290L-CDR1
KSSQSLLHSDGKTYLN

SEQ ID NO: 151 - protein, 7 aa, Artificial Sequence
  H2M290L-CDR2
LVSNLDS

SEQ ID NO: 152 - protein, 8 aa, Artificial Sequence
  H2M290L-CDR3
WQGTHFPT

SEQ ID NO: 153 - protein, 5 aa, Artificial Sequence
  H2M291H-CDR1
GYTMN

SEQ ID NO: 154 - protein, 17 aa, Artificial Sequence
  H2M291H-CDR2
LINPYNGNTRYNQKFQD

SEQ ID NO: 155 - protein, 5 aa, Artificial Sequence
  H2M291H-CDR3
EPSDY

SEQ ID NO: 156 - protein, 16 aa, Artificial Sequence
  H2M291L-CDR1
RSSQSLVHINGNTYLH

SEQ ID NO: 157 - protein, 7 aa, Artificial Sequence
  H2M291L-CDR2
KVSKRFS

SEQ ID NO: 158 - protein, 9 aa, Artificial Sequence
  H2M291L-CDR3
SQSTHVPPT

SEQ ID NO: 159 - protein, 5 aa, Artificial Sequence
  H2M292H-CDR1
GYTMN

SEQ ID NO: 160 - protein, 17 aa, Artificial Sequence
  H2M292H-CDR2
LINPSNGGTRYNQKFKD

SEQ ID NO: 161 - protein, 5 aa, Artificial Sequence
  H2M292H-CDR3
EPSDY

SEQ ID NO: 162 - protein, 16 aa, Artificial Sequence
  H2M292L-CDR1
RSSQSLVHSNGNTYLH

SEQ ID NO: 163 - protein, 7 aa, Artificial Sequence
  H2M292L-CDR2
KVSNRFS

SEQ ID NO: 164 - protein, 9 aa, Artificial Sequence
  H2M292L-CDR3
SQSTHVPPT

SEQ ID NO: 165 - protein, 5 aa, Artificial Sequence
  H2M293H-CDR1
NYGIF

SEQ ID NO: 166 - protein, 17 aa, Artificial Sequence
  H2M293H-CDR2
TVKSNGGSTYYPDSVKG

SEQ ID NO: 167 - protein, 5 aa, Artificial Sequence
  H2M293H-CDR3
EGGDY

SEQ ID NO: 168 - protein, 11 aa, Artificial Sequence
  H2M293L-CDR1
KASQDVGTAVA

SEQ ID NO: 169 - protein, 7 aa, Artificial Sequence
  H2M293L-CDR2
WTSTRHI

SEQ ID NO: 170 - protein, 9 aa, Artificial Sequence
  H2M293L-CDR3
QQYSKNPLT

SEQ ID NO: 171 - protein, 5 aa, Artificial Sequence
  H2M294H-CDR1
SYGMS

SEQ ID NO: 172 - protein, 17 aa, Artificial Sequence
  H2M294H-CDR2
TINSNGGGTYYPDSVKG

SEQ ID NO: 173 - protein, 7 aa, Artificial Sequence
  H2M294H-CDR3
PGSWFPY

SEQ ID NO: 174 - protein, 16 aa, Artificial Sequence
  H2M294L-CDR1
KSSQSLLDSDGKTYLH

SEQ ID NO: 175 - protein, 7 aa, Artificial Sequence
  H2M294L-CDR2
LVSKLDS

SEQ ID NO: 176 - protein, 9 aa, Artificial Sequence
  H2M294L-CDR3
WQGTHFPQT

SEQ ID NO: 177 - protein, 5 aa, Artificial Sequence
  H2M295H-CDR1
GYTMN

SEQ ID NO: 178 - protein, 17 aa, Artificial Sequence
  H2M295H-CDR2
LINPYNGGTRYNQKFKG

SEQ ID NO: 179 - protein, 5 aa, Artificial Sequence
  H2M295H-CDR3
EPSDY

SEQ ID NO: 180 - protein, 16 aa, Artificial Sequence
  H2M295L-CDR1
RSSQSLVHSNGNTYLH

SEQ ID NO: 181 - protein, 7 aa, Artificial Sequence
  H2M295L-CDR2
KVSKRFS

SEQ ID NO: 182 - protein, 9 aa, Artificial Sequence
  H2M295L-CDR3
SQSSHVPPT

SEQ ID NO: 183 - protein, 7 aa, Artificial Sequence
  H2M296H-CDR1
TSGMGVG

SEQ ID NO: 184 - protein, 16 aa, Artificial Sequence
  H2M296H-CDR2
HIWWDDDKRYNPALKS

SEQ ID NO: 185 - protein, 9 aa, Artificial Sequence
  H2M296H-CDR3
IEGQRGFAY

SEQ ID NO: 186 - protein, 17 aa, Artificial Sequence
  H2M296L-CDR1
KSSQSLLYSRNQKNYLA

SEQ ID NO: 187 - protein, 7 aa, Artificial Sequence
  H2M296L-CDR2
WASTRES

SEQ ID NO: 188 - protein, 9 aa, Artificial Sequence
  H2M296L-CDR3
QQYYSQPYT

SEQ ID NO: 189 - protein, 5 aa, Artificial Sequence
  H2M297H-CDR1
SYGIF

SEQ ID NO: 190 - protein, 17 aa, Artificial Sequence
  H2M297H-CDR2
TIKSNGGRTYYPDSVKG

SEQ ID NO: 191 - protein, 5 aa, Artificial Sequence
  H2M297H-CDR3
EGGDY

SEQ ID NO: 192 - protein, 16 aa, Artificial Sequence
  H2M297L-CDR1
RSSQSVVHSNGNTYLE

SEQ ID NO: 193 - protein, 7 aa, Artificial Sequence
  H2M297L-CDR2
KVSNRFS

SEQ ID NO: 194 - protein, 9 aa, Artificial Sequence
  H2M297L-CDR3
FQGSRVPPT

SEQ ID NO: 195 - protein, 5 aa, Artificial Sequence
  H2M298H-CDR1
RYSMS

SEQ ID NO: 196 - protein, 17 aa, Artificial Sequence
  H2M298H-CDR2
IISTGGSYMFYPDSAKG

SEQ ID NO: 197 - protein, 5 aa, Artificial Sequence
  H2M298H-CDR3
EAGDY

SEQ ID NO: 198 - protein, 16 aa, Artificial Sequence
  H2M298L-CDR1
KSSQSLLHSDGKTYLN

SEQ ID NO: 199 - protein, 7 aa, Artificial Sequence
  H2M298L-CDR2
LVSKLDS

SEQ ID NO: 200 - protein, 8 aa, Artificial Sequence
  H2M298L-CDR3
WQGTHFPT

SEQ ID NO: 201 - protein, 5 aa, Artificial Sequence
  H2M299H-CDR1
IYGIF

SEQ ID NO: 202 - protein, 17 aa, Artificial Sequence
  H2M299H-CDR2
TIHSNGGRIYYPDSVKG

SEQ ID NO: 203 - protein, 5 aa, Artificial Sequence
  H2M299H-CDR3
EGGDY

SEQ ID NO: 204 - protein, 11 aa, Artificial Sequence
  H2M299L-CDR1
KASQDVGTAVA

SEQ ID NO: 205 - protein, 7 aa, Artificial Sequence
  H2M299L-CDR2
WASTRHT

SEQ ID NO: 206 - protein, 9 aa, Artificial Sequence
  H2M299L-CDR3
QQYRRYPLT